European Patent Specification EP 4 314 340 B1, published April 22, 2026. Title: COMPOSITIONS AND METHODS FOR SIMULTANEOUS GENETIC ANALYSIS OF MULTIPLE LIBRARIES. Applicant: Resolution Bioscience, Inc. The sequence listing filed with the application follows.

SEQUENCE LISTING (83 sequences)

SEQ ID NO: 1 - DNA, 10 bp, Artificial Sequence
  Exemplary Anchor 1
acgtatgcca

SEQ ID NO: 2 - DNA, 10 bp, Artificial Sequence
  Exemplary Anchor 2
ctagcgttac

SEQ ID NO: 3 - DNA, 10 bp, Artificial Sequence
  Exemplary Anchor 3
gatcgacatg

SEQ ID NO: 4 - DNA, 10 bp, Artificial Sequence
  Exemplary Anchor 4
tgcatcaggt

SEQ ID NO: 5 - DNA, 25 bp, Artificial Sequence
  Library Primer (single amplification primer; AKA primer)
tgcaggaccagagaattcgaataca

SEQ ID NO: 6 - DNA, 47 bp, Artificial Sequence
  exemplary partner oligonucleotide
  misc_feature (47)..(47): Biotin-TEG label attached
gtgaaaaccaggatcaactcccgtgccagtcacatctcagatgagct

SEQ ID NO: 7 - DNA, 58 bp, Artificial Sequence
  Forward Primer (Post Hyb Primer mix/Genomic Mix F/Primer F)
aatgatacggcgaccaccgagatctacacgtcatgcaggaccagagaattcgaataca

SEQ ID NO: 8 - DNA, 57 bp, Artificial Sequence
  Reverse Primer 63
caagcagaagacggcatacgagatgtgactggcacgggaccagagaattcgaataca

SEQ ID NO: 9 - DNA, 57 bp, Artificial Sequence
  Reverse Primer LPWG_AMP_R (Genomic Mix R)
caagcagaagacggcatacgagatgtgactggtgcaggaccagagaattcgaataca

SEQ ID NO: 10 - DNA, 57 bp, Artificial Sequence; identical to SEQ ID NO: 8
  Seq Forward Primer (FWD Seq Primer)

SEQ ID NO: 11 - DNA, 33 bp, Artificial Sequence
  Seq Reverse Primer 62 (REV Seq Primer)
gtgactggcacgggaccagagaattcgaataca

SEQ ID NO: 12 - DNA, 33 bp, Artificial Sequence
  Reverse Primer LPWG_SEQ_R:
gtgactggtgcaggaccagagaattcgaataca

SEQ ID NO: 13 - DNA, 20 bp, Artificial Sequence
  Oligo 1 (Genomic Mix):
aatgatacggcgaccaccga

SEQ ID NO: 14 - DNA, 21 bp, Artificial Sequence
  Oligo 2 (Genomic Mix):
caagcagaagacggcatacga

SEQ ID NO: 15 - DNA, 20 bp, Artificial Sequence
  Oligo 1c:
tcggtggtcgccgtatcatt

SEQ ID NO: 16 - DNA, 21 bp, Artificial Sequence
  Oligo 2c:
tcgtatgccgtcttctgcttg

SEQ ID NO: 17 - DNA, 17 bp, Artificial Sequence
  Empty read tag
ggggggggggggggggg

SEQ ID NO: 18 - DNA, 10 bp, Artificial Sequence
  non-ligation-anchor region 1
tggcatacgt

SEQ ID NO: 19 - DNA, 10 bp, Artificial Sequence
  non-ligation-anchor region 2
gtaacgctag

SEQ ID NO: 20 - DNA, 10 bp, Artificial Sequence
  non-ligation-anchor region 3
catgtcgatc

SEQ ID NO: 21 - DNA, 10 bp, Artificial Sequence
  non-ligation-anchor region 4
acctgatgca

SEQ ID NO: 22 - DNA, 47 bp, Artificial Sequence
  exemplary ligation strand 1
  misc_feature (34)..(36): n is a, c, g, or t
tgcaggaccagagaattcgaatacaaaaatcctnnnacgtatgccat

SEQ ID NO: 23 - DNA, 47 bp, Artificial Sequence
  exemplary ligation strand 2
  misc_feature (34)..(36): n is a, c, g, or t
tgcaggaccagagaattcgaatacaaatgatctnnnacgtatgccat

SEQ ID NO: 24 - DNA, 47 bp, Artificial Sequence
  exemplary ligation strand 3
  misc_feature (34)..(36): n is a, c, g, or t
tgcaggaccagagaattcgaatacaagtaatagnnnacgtatgccat

SEQ ID NO: 25 - DNA, 47 bp, Artificial Sequence
  exemplary ligation strand 4
  misc_feature (34)..(36): n is a, c, g, or t
tgcaggaccagagaattcgaatacacacctccgnnnacgtatgccat

SEQ ID NO: 26 - DNA, 47 bp, Artificial Sequence
  exemplary ligation strand 5
  misc_feature (34)..(36): n is a, c, g, or t
tgcaggaccagagaattcgaatacacgccccatnnnacgtatgccat

SEQ ID NO: 27 - DNA, 47 bp, Artificial Sequence
  exemplary ligation strand 6
  misc_feature (34)..(36): n is a, c, g, or t
tgcaggaccagagaattcgaatacactaccaagnnnacgtatgccat

SEQ ID NO: 28 - DNA, 47 bp, Artificial Sequence
  exemplary ligation strand 7
  misc_feature (34)..(36): n is a, c, g, or t
tgcaggaccagagaattcgaatacactgtcgttnnnacgtatgccat

SEQ ID NO: 29 - DNA, 47 bp, Artificial Sequence
  exemplary ligation strand 8
  misc_feature (34)..(36): n is a, c, g, or t
tgcaggaccagagaattcgaatacagcaaatggnnnacgtatgccat

SEQ ID NO: 30 - DNA, 47 bp, Artificial Sequence
  exemplary ligation strand 9
  misc_feature (34)..(36): n is a, c, g, or t
tgcaggaccagagaattcgaatacagctcgagcnnnacgtatgccat

SEQ ID NO: 31 - DNA, 47 bp, Artificial Sequence
  exemplary ligation strand 10
  misc_feature (34)..(36): n is a, c, g, or t
tgcaggaccagagaattcgaatacagtccacaannnacgtatgccat

SEQ ID NO: 32 - DNA, 47 bp, Artificial Sequence
  exemplary ligation strand 11
  misc_feature (34)..(36): n is a, c, g, or t
tgcaggaccagagaattcgaatacagttaccctnnnacgtatgccat

SEQ ID NO: 33 - DNA, 47 bp, Artificial Sequence
  exemplary ligation strand 12
  misc_feature (34)..(36): n is a, c, g, or t
tgcaggaccagagaattcgaatacatagttttcnnnacgtatgccat

SEQ ID NO: 34 - DNA, 47 bp, Artificial Sequence
  exemplary ligation strand 13
  misc_feature (34)..(36): n is a, c, g, or t
tgcaggaccagagaattcgaatacatctcagagnnnacgtatgccat

SEQ ID NO: 35 - DNA, 47 bp, Artificial Sequence
  exemplary ligation strand 14
  misc_feature (34)..(36): n is a, c, g, or t
tgcaggaccagagaattcgaatacatgaccttcnnnacgtatgccat

SEQ ID NO: 36 - DNA, 47 bp, Artificial Sequence
  exemplary ligation strand 15
  misc_feature (34)..(36): n is a, c, g, or t
tgcaggaccagagaattcgaatacattacggcannnacgtatgccat

SEQ ID NO: 37 - DNA, 47 bp, Artificial Sequence
  exemplary ligation strand 16
  misc_feature (34)..(36): n is a, c, g, or t
tgcaggaccagagaattcgaatacaaacaaaacnnntgcatcaggtt

SEQ ID NO: 38 - DNA, 47 bp, Artificial Sequence
  exemplary ligation strand 17
  misc_feature (34)..(36): n is a, c, g, or t
tgcaggaccagagaattcgaatacaacactgcannntgcatcaggtt

SEQ ID NO: 39 - DNA, 47 bp, Artificial Sequence
  exemplary ligation strand 18
  misc_feature (34)..(36): n is a, c, g, or t
tgcaggaccagagaattcgaatacaatcgcgatnnntgcatcaggtt

SEQ ID NO: 40 - DNA, 47 bp, Artificial Sequence
  exemplary ligation strand 19
  misc_feature (34)..(36): n is a, c, g, or t
tgcaggaccagagaattcgaatacaatggtggannntgcatcaggtt

SEQ ID NO: 41 - DNA, 47 bp, Artificial Sequence
  exemplary ligation strand 20
  misc_feature (34)..(36): n is a, c, g, or t
tgcaggaccagagaattcgaatacacaactctcnnntgcatcaggtt

SEQ ID NO: 42 - DNA, 47 bp, Artificial Sequence
  exemplary ligation strand 21
  misc_feature (34)..(36): n is a, c, g, or t
tgcaggaccagagaattcgaatacacgcccgaannntgcatcaggtt

SEQ ID NO: 43 - DNA, 47 bp, Artificial Sequence
  exemplary ligation strand 22
  misc_feature (34)..(36): n is a, c, g, or t
tgcaggaccagagaattcgaatacacgtatgacnnntgcatcaggtt

SEQ ID NO: 44 - DNA, 47 bp, Artificial Sequence
  exemplary ligation strand 23
  misc_feature (34)..(36): n is a, c, g, or t
tgcaggaccagagaattcgaatacagaaacgacnnntgcatcaggtt

SEQ ID NO: 45 - DNA, 47 bp, Artificial Sequence
  exemplary ligation strand 24
  misc_feature (34)..(36): n is a, c, g, or t
tgcaggaccagagaattcgaatacagactctgannntgcatcaggtt

SEQ ID NO: 46 - DNA, 47 bp, Artificial Sequence
  exemplary ligation strand 25
  misc_feature (34)..(36): n is a, c, g, or t
tgcaggaccagagaattcgaatacagtcactctnnntgcatcaggtt

SEQ ID NO: 47 - DNA, 47 bp, Artificial Sequence
  exemplary ligation strand 26
  misc_feature (34)..(36): n is a, c, g, or t
tgcaggaccagagaattcgaatacatactggacnnntgcatcaggtt

SEQ ID NO: 48 - DNA, 47 bp, Artificial Sequence
  exemplary ligation strand 27
  misc_feature (34)..(36): n is a, c, g, or t
tgcaggaccagagaattcgaatacatgcgatacnnntgcatcaggtt

SEQ ID NO: 49 - DNA, 47 bp, Artificial Sequence
  exemplary ligation strand 28
  misc_feature (34)..(36): n is a, c, g, or t
tgcaggaccagagaattcgaatacatgttaatgnnntgcatcaggtt

SEQ ID NO: 50 - DNA, 47 bp, Artificial Sequence
  exemplary ligation strand 29
  misc_feature (34)..(36): n is a, c, g, or t
tgcaggaccagagaattcgaatacattgtacttnnntgcatcaggtt

SEQ ID NO: 51 - DNA, 47 bp, Artificial Sequence
  exemplary ligation strand 30
  misc_feature (34)..(36): n is a, c, g, or t
tgcaggaccagagaattcgaatacatttggctcnnntgcatcaggtt

SEQ ID NO: 52 - DNA, 47 bp, Artificial Sequence
  exemplary ligation strand 31
  misc_feature (34)..(36): n is a, c, g, or t
tgcaggaccagagaattcgaatacaaacgcctannngatcgacatgt

SEQ ID NO: 53 - DNA, 47 bp, Artificial Sequence
  exemplary ligation strand 32
  misc_feature (34)..(36): n is a, c, g, or t
tgcaggaccagagaattcgaatacaaagtttcannngatcgacatgt

SEQ ID NO: 54 - DNA, 47 bp, Artificial Sequence
  exemplary ligation strand 33
  misc_feature (34)..(36): n is a, c, g, or t
tgcaggaccagagaattcgaatacaacagcgaannngatcgacatgt

SEQ ID NO: 55 - DNA, 47 bp, Artificial Sequence
  exemplary ligation strand 34
  misc_feature (34)..(36): n is a, c, g, or t
tgcaggaccagagaattcgaatacaagcgcctgnnngatcgacatgt

SEQ ID NO: 56 - DNA, 47 bp, Artificial Sequence
  exemplary ligation strand 35
  misc_feature (34)..(36): n is a, c, g, or t
tgcaggaccagagaattcgaatacacaacccttnnngatcgacatgt

SEQ ID NO: 57 - DNA, 47 bp, Artificial Sequence
  exemplary ligation strand 36
  misc_feature (34)..(36): n is a, c, g, or t
tgcaggaccagagaattcgaatacacagaataannngatcgacatgt

SEQ ID NO: 58 - DNA, 47 bp, Artificial Sequence
  exemplary ligation strand 37
  misc_feature (34)..(36): n is a, c, g, or t
tgcaggaccagagaattcgaatacacggacaccnnngatcgacatgt

SEQ ID NO: 59 - DNA, 47 bp, Artificial Sequence
  exemplary ligation strand 38
  misc_feature (34)..(36): n is a, c, g, or t
tgcaggaccagagaattcgaatacagcctattcnnngatcgacatgt

SEQ ID NO: 60 - DNA, 47 bp, Artificial Sequence
  exemplary ligation strand 39
  misc_feature (34)..(36): n is a, c, g, or t
tgcaggaccagagaattcgaatacagcgtccagnnngatcgacatgt

SEQ ID NO: 61 - DNA, 47 bp, Artificial Sequence
  exemplary ligation strand 40
  misc_feature (34)..(36): n is a, c, g, or t
tgcaggaccagagaattcgaatacaggtacaagnnngatcgacatgt

SEQ ID NO: 62 - DNA, 47 bp, Artificial Sequence
  exemplary ligation strand 41
  misc_feature (34)..(36): n is a, c, g, or t
tgcaggaccagagaattcgaatacataaccctcnnngatcgacatgt

SEQ ID NO: 63 - DNA, 47 bp, Artificial Sequence
  exemplary ligation strand 42
  misc_feature (34)..(36): n is a, c, g, or t
tgcaggaccagagaattcgaatacataggagtgnnngatcgacatgt

SEQ ID NO: 64 - DNA, 47 bp, Artificial Sequence
  exemplary ligation strand 43
  misc_feature (34)..(36): n is a, c, g, or t
tgcaggaccagagaattcgaatacatccgcattnnngatcgacatgt

SEQ ID NO: 65 - DNA, 47 bp, Artificial Sequence
  exemplary ligation strand 44
  misc_feature (34)..(36): n is a, c, g, or t
tgcaggaccagagaattcgaatacatgcgtcaannngatcgacatgt

SEQ ID NO: 66 - DNA, 47 bp, Artificial Sequence
  exemplary ligation strand 45
  misc_feature (34)..(36): n is a, c, g, or t
tgcaggaccagagaattcgaatacattggtaatnnngatcgacatgt

SEQ ID NO: 67 - DNA, 47 bp, Artificial Sequence
  exemplary ligation strand 46
  misc_feature (34)..(36): n is a, c, g, or t
tgcaggaccagagaattcgaatacaaatagcttnnnctagcgttact

SEQ ID NO: 68 - DNA, 47 bp, Artificial Sequence
  exemplary ligation strand 47
  misc_feature (34)..(36): n is a, c, g, or t
tgcaggaccagagaattcgaatacaagagagagnnnctagcgttact

SEQ ID NO: 69 - DNA, 47 bp, Artificial Sequence
  exemplary ligation strand 48
  misc_feature (34)..(36): n is a, c, g, or t
tgcaggaccagagaattcgaatacacaacctgannnctagcgttact

SEQ ID NO: 70 - DNA, 47 bp, Artificial Sequence
  exemplary ligation strand 49
  misc_feature (34)..(36): n is a, c, g, or t
tgcaggaccagagaattcgaatacacatatggcnnnctagcgttact

SEQ ID NO: 71 - DNA, 47 bp, Artificial Sequence
  exemplary ligation strand 50
  misc_feature (34)..(36): n is a, c, g, or t
tgcaggaccagagaattcgaatacaccatatccnnnctagcgttact

SEQ ID NO: 72 - DNA, 47 bp, Artificial Sequence
  exemplary ligation strand 51
  misc_feature (34)..(36): n is a, c, g, or t
tgcaggaccagagaattcgaatacacgaggtccnnnctagcgttact

SEQ ID NO: 73 - DNA, 47 bp, Artificial Sequence
  exemplary ligation strand 52
  misc_feature (34)..(36): n is a, c, g, or t
tgcaggaccagagaattcgaatacacgtcaatgnnnctagcgttact

SEQ ID NO: 74 - DNA, 47 bp, Artificial Sequence
  exemplary ligation strand 53
  misc_feature (34)..(36): n is a, c, g, or t
tgcaggaccagagaattcgaatacacttatcatnnnctagcgttact

SEQ ID NO: 75 - DNA, 47 bp, Artificial Sequence
  exemplary ligation strand 54
  misc_feature (34)..(36): n is a, c, g, or t
tgcaggaccagagaattcgaatacagcattgacnnnctagcgttact

SEQ ID NO: 76 - DNA, 47 bp, Artificial Sequence
  exemplary ligation strand 55
  misc_feature (34)..(36): n is a, c, g, or t
tgcaggaccagagaattcgaatacaggaggtatnnnctagcgttact

SEQ ID NO: 77 - DNA, 47 bp, Artificial Sequence
  exemplary ligation strand 56
  misc_feature (34)..(36): n is a, c, g, or t
tgcaggaccagagaattcgaatacataacagttnnnctagcgttact

SEQ ID NO: 78 - DNA, 47 bp, Artificial Sequence
  exemplary ligation strand 57
  misc_feature (34)..(36): n is a, c, g, or t
tgcaggaccagagaattcgaatacatcgaacacnnnctagcgttact

SEQ ID NO: 79 - DNA, 47 bp, Artificial Sequence
  exemplary ligation strand 58
  misc_feature (34)..(36): n is a, c, g, or t
tgcaggaccagagaattcgaatacatgcataatnnnctagcgttact

SEQ ID NO: 80 - DNA, 47 bp, Artificial Sequence
  exemplary ligation strand 59
  misc_feature (34)..(36): n is a, c, g, or t
tgcaggaccagagaattcgaatacatgtcataannnctagcgttact

SEQ ID NO: 81 - DNA, 47 bp, Artificial Sequence
  exemplary ligation strand 60
  misc_feature (34)..(36): n is a, c, g, or t
tgcaggaccagagaattcgaatacattgcgcggnnnctagcgttact

SEQ ID NO: 82 - DNA, 57 bp, Artificial Sequence
  Reverse Primer (Post Hyb Primer mix)
caagcagaagacggcatacgagatgtgactggcacgggagttgatcctggttttcac

SEQ ID NO: 83 - DNA, 33 bp, Artificial Sequence
  Index sequencing primer
tgtattcgaattctctggtcccgtgccagtcac